European Patent Application EP 4 303 314 A2, published January 10, 2024. Title: POLYPEPTIDE TAGGED NUCLEOTIDES AND USE THEREOF IN NUCLEIC ACID SEQUENCING BY NANOPORE DETECTION. Applicant: F. Hoffmann-La Roche AG. Application EP, filed August 26, 2016. The sequence listing filed with the application follows.

SEQUENCE LISTING (24 sequences)

SEQ ID NO: 1 - protein, 69 aa, synthetic construct
  REGION 1..69: note = artificial
EAAAEAAAEAAAEAAAEAAAEAAAEAAAEAAAEAAAEAAAEAAAEAAAEAAAEAAAEAAAEAAAEEEEE

SEQ ID NO: 2 - protein, 57 aa, synthetic construct
  REGION 1..57: note = Synthetic peptide
EAAAEAAAEAAAEAAAEAAAEAAAEAAAEAAAEAAAEAAAEAAAEAAAEAAAEEEEE

SEQ ID NO: 3 - protein, 45 aa, synthetic construct
  REGION 1..45: note = synthetic peptide
EAAAEAAAEAAAEAAAEAAAEAAAEAAAEAAAEAAAEAAAEEEEE

SEQ ID NO: 4 - protein, 69 aa, synthetic construct
  REGION 1..69: note = synthetic peptide
EAAAEAAAEAAAEAAAEAAAEAAAEAAAEAAAEAAAEAAAEAAAEAAAEAAAEAAAEAAAEAAAGGGGE

SEQ ID NO: 5 - protein, 50 aa, synthetic construct
  REGION 1..50: note = synthetic peptide
AEAEAEAEAEAEAEAEAEAEAEAEAEAEAEAEAEAEAEAEAEAEAEAEAE

SEQ ID NO: 6 - protein, 70 aa, synthetic construct
  REGION 1..70: note = synthetic peptide
EAAAEAAAEAAAEAAAEAAAEAAAEAAAEAAAPEAAAEAAAEAAAEAAAEAAAEAAAEAAAEAAAEEEEE

SEQ ID NO: 7 - protein, 72 aa, synthetic construct
  REGION 1..72: note = synthetic peptide
EAAAEAAAEAAAEAAAPEAAAEAAAEAAAEAAAPEAAAEAAAEAAAEAAAPEAAAEAAAEAAAEAAAEEEEE

SEQ ID NO: 8 - protein, 69 aa, synthetic construct
  REGION 1..69: note = synthetic peptide
EAAAKAAAEAAAKAAAEAAAKAAAEAAAKAAAEAAAEAAAEAAAEAAAEAAAEAAAEAAAEAAAEEEEE

SEQ ID NO: 9 - protein, 69 aa, synthetic construct
  REGION 1..69: note = synthetic peptide
EAAAKAAAEAAAKAAAEAAAKAAAEAAAKAAAEAAAKAAAEAAAKAAAEAAAKAAAEAAAKAAAEEEEE

SEQ ID NO: 10 - protein, 55 aa, synthetic construct
  REGION 1..55: note = synthetic peptide
EPPPPPPPPPEPPPPPPPPPEPPPPPPPPPEPPPPPPPPPEPPPPPPPPPEEEEE

SEQ ID NO: 11 - protein, 69 aa, synthetic construct
  REGION 1..69: note = synthetic peptide
EPPPEPPPEPPPEPPPEPPPEPPPEPPPEPPPEPPPEPPPEPPPEPPPEPPPEPPPEPPPEPPPEEEEE

SEQ ID NO: 12 - protein, 50 aa, synthetic construct
  REGION 1..50: note = synthetic peptide
PPPPPPPPPPPPPPPPPPPPPPPPPPPPPPPPPPPPPPPPPPPPPEEEEE

SEQ ID NO: 13 - protein, 69 aa, synthetic construct
  REGION 1..69: note = synthetic peptide
RAAARAAARAAARAAARAAARAAARAAARAAARAAARAAARAAARAAARAAARAAARAAARAAARRRRR

SEQ ID NO: 14 - protein, 69 aa, synthetic construct
  REGION 1..69: note = synthetic peptide
EATAEATAEATAEATAEATAEATAEATAEATAEATAEATAEATAEATAEATAEATAEATAEATAEEEEE

SEQ ID NO: 15 - protein, 70 aa, synthetic construct
  REGION 1..70: note = synthetic peptide
GEAAAEAAAEAAAEAAAEAAAEAAAEAAAEAAAEAAAEAAAEAAAEAAAEAAAEAAAEAAAEAAAEEEEE

SEQ ID NO: 16 - protein, 58 aa, synthetic construct
  REGION 1..58: note = synthetic peptide
GEAAAEAAAEAAAEAAAEAAAEAAAEAAAEAAAEAAAEAAAEAAAEAAAEAAAEEEEE

SEQ ID NO: 17 - protein, 46 aa, synthetic construct
  REGION 1..46: note = synthetic peptide
GEAAAEAAAEAAAEAAAEAAAEAAAEAAAEAAAEAAAEAAAEEEEE

SEQ ID NO: 18 - protein, 71 aa, synthetic construct
  REGION 1..71: note = synthetic peptide
GEAAAEAAAEAAAEAAAEAAAEAAAEAAAEAAAPEAAAEAAAEAAAEAAAEAAAEAAAEAAAEAAAEEEEE

SEQ ID NO: 19 - protein, 51 aa, synthetic construct
  REGION 1..51: note = synthetic peptide
AEAEAEAEAEAEAEAEAEAEAEAEAEAEAEAEAEAEAEAEAEAEAEAEAEK

SEQ ID NO: 20 - protein, 73 aa, synthetic construct
  REGION 1..73: note = synthetic peptide
GEAAAEAAAEAAAEAAAPEAAAEAAAEAAAEAAAPEAAAEAAAEAAAEAAAPEAAAEAAAEAAAEAAAEEEEE

SEQ ID NO: 21 - protein, 70 aa, synthetic construct
  REGION 1..70: note = synthetic peptide
GEAAAKAAAEAAAKAAAEAAAKAAAEAAAKAAAEAAAEAAAEAAAEAAAEAAAEAAAEAAAEAAAEEEEE

SEQ ID NO: 22 - protein, 70 aa, synthetic construct
  REGION 1..70: note = synthetic peptide
GEAAAKAAAEAAAKAAAEAAAKAAAEAAAKAAAEAAAKAAAEAAAKAAAEAAAKAAAEAAAKAAAEEEEE

SEQ ID NO: 23 - protein, 70 aa, synthetic construct
  REGION 1..70: note = synthetic peptide
GEPPPEPPPEPPPEPPPEPPPEPPPEPPPEPPPEPPPEPPPEPPPEPPPEPPPEPPPEPPPEPPPEEEEE

SEQ ID NO: 24 - protein, 70 aa, synthetic construct; identical to SEQ ID NO: 15
  REGION 1..70: note = synthetic peptide